European Patent Application EP 4 289 865 A1, published December 13, 2023. Title: ANTI-TNFR2 ANTIBODY AND USE THEREOF. Applicant: Innovent Biologics (Suzhou) Co., Ltd. The sequence listing filed with the application follows.

SEQUENCE LISTING (69 sequences)

SEQ ID NO: 1 - protein, 10 aa, artificial sequence
  synthetic
DYSFTNYYIH

SEQ ID NO: 2 - protein, 17 aa, artificial sequence
  synthetic
WIYPGNVITKYHEKFKG

SEQ ID NO: 3 - protein, 9 aa, artificial sequence
  synthetic
SRATGYFDY

SEQ ID NO: 4 - protein, 11 aa, artificial sequence
  synthetic
RASQDIRNYLN

SEQ ID NO: 5 - protein, 7 aa, artificial sequence
  synthetic
YTSRLHS

SEQ ID NO: 6 - protein, 9 aa, artificial sequence
  synthetic
QQFNTLPWT

SEQ ID NO: 7 - protein, 10 aa, artificial sequence
  synthetic
GYTFTSYWMQ

SEQ ID NO: 8 - protein, 17 aa, artificial sequence
  synthetic
AIYPGDGDTRYTQKFKG

SEQ ID NO: 9 - protein, 10 aa, artificial sequence
  synthetic
DDGLYYAMDY

SEQ ID NO: 10 - protein, 12 aa, artificial sequence
  synthetic
TASSSVSSSYLH

SEQ ID NO: 11 - protein, 7 aa, artificial sequence
  synthetic
STSNLAS

SEQ ID NO: 12 - protein, 9 aa, artificial sequence
  synthetic
HQYHRSPPT

SEQ ID NO: 13 - protein, 10 aa, artificial sequence
  synthetic
GYTFTDYSMN

SEQ ID NO: 14 - protein, 17 aa, artificial sequence
  synthetic
WLNTETGEPIYADDFKG

SEQ ID NO: 15 - protein, 13 aa, artificial sequence
  synthetic
EAIYYGTSYVLDY

SEQ ID NO: 16 - protein, 15 aa, artificial sequence
  synthetic
RASESVEYYGTNFMQ

SEQ ID NO: 17 - protein, 7 aa, artificial sequence
  synthetic
SASNVES

SEQ ID NO: 18 - protein, 9 aa, artificial sequence
  synthetic
QQSRKDPST

SEQ ID NO: 19 - protein, 118 aa, artificial sequence
  synthetic
QVQLQQSGPELVKPGASVTISCKASDYSFTNYYIHWVKQRPGQGLEWIGWIYPGNVITKYHEKFKGKAILTADTSSTTAYMQLNSLTSEDSAVYFCARSRATGYFDYWGQGTTLTVSS

SEQ ID NO: 20 - protein, 107 aa, artificial sequence
  synthetic
DIQMTQTTSSLSASLGDRVTISCRASQDIRNYLNWFQQKPDGTIKLLIYYTSRLHSGVPSRFSGSGSGTDYSLTISNLEQEDMATYFCQQFNTLPWTFGGGTKLEIK

SEQ ID NO: 21 - protein, 118 aa, artificial sequence
  synthetic
QVQLVQSGAEVKKPGASVKVSCKASDYSFTNYYIHWVRQAPGQGLEWMGWIYPGNVITKYHEKFKGRVTMTADTSTSTAYMELSSLRSEDTAVYYCARSRATGYFDYWGQGTLVTVSS

SEQ ID NO: 22 - protein, 107 aa, artificial sequence
  synthetic
DIQMTQSPSSLSASVGDRVTITCRASQDIRNYLNWYQQKPGKAPKLLIYYTSRLHSGVPSRFSGSGSGTDYTLTISSLQPEDFATYYCQQFNTLPWTFGGGTKVEIK

SEQ ID NO: 23 - protein, 119 aa, artificial sequence
  synthetic
EVQLQQSGAELARPGASVMLSCKASGYTFTSYWMQWLKQRPGQGLEWIGAIYPGDGDTRYTQKFKGKATLTADKSSSTAYMQLSSLASEDSAVYYCVRDDGLYYAMDYWGQGTSVTVSS

SEQ ID NO: 24 - protein, 108 aa, artificial sequence
  synthetic
QIVLTQSPTIMSASLGERVTMTCTASSSVSSSYLHWYQQKPGSSPKLWIYSTSNLASGVPARFSGSGSGTSYSLTISSMEAEDAATYYCHQYHRSPPTFGGGTKLEIK

SEQ ID NO: 25 - protein, 122 aa, artificial sequence
  synthetic
QIQLVQSGPELKKPGETVKISCKASGYTFTDYSMNWVKQAPGKGLKWMGWLNTETGEPIYADDFKGRFVFSLETSASTAYLEINNLNDEDTATYFCAREAIYYGTSYVLDYWGQGTSVTVSS

SEQ ID NO: 26 - protein, 111 aa, artificial sequence
  synthetic
DIVLTQSPASLAVSLGQRATISCRASESVEYYGTNFMQWYQQKPGQPPKLLIYSASNVESGVPARFSGSGSGTDFSLNIHPVEEDDIAVYFCQQSRKDPSTFGEGTNLEIK

SEQ ID NO: 27 - protein, 122 aa, artificial sequence
  synthetic
QIQLVQSGSELKKPGASVKVSCKASGYTFTDYSMNWVRQAPGQGLEWMGWLNTETGEPIYADDFKGRFVFSLDTSVSTAYLQISSLKAEDTAVYFCAREAIYYGTSYVLDYWGQGTLVTVSS

SEQ ID NO: 28 - protein, 111 aa, artificial sequence
  synthetic
DIVLTQSPASLAVSPGQRATITCRASESVEYYGTNFMQWYQQKPGQPPKLLIYSASNVESGVPARFSGSGSGTDFTLTINPVEANDTANYYCQQSRKDPSTFGQGTKLEIK

SEQ ID NO: 29 - protein, 122 aa, artificial sequence
  synthetic
QVQLVQSGAEVKKPGASVKVSCKASGYTFTDYSMNWVRQAPGQRLEWMGWLNTETGEPIYADDFKGRVTITRDTSASTAYMELSSLRSEDTAVYYCAREAIYYGTSYVLDYWGQGTLVTVSS

SEQ ID NO: 30 - protein, 111 aa, artificial sequence
  synthetic
DIVLTQSPASLAVSPGQRATITCRASESVEYYGTNFMQWYQQKPGQPPKLLIYSASNVESGVPARFSGSGSGTDFTLTINPVEANDTANYFCQQSRKDPSTFGQGTKLEIK

SEQ ID NO: 31 - protein, 111 aa, artificial sequence
  synthetic
DIVLTQSPASLAVSPGQRATITCRASESVEYYGTNFMQWYQQKPGQPPKLLIYSASNVESGVPARFSGSGSGTDFTLTINPVEAQDTANYFCQQSRKDPSTFGQGTKLEIK

SEQ ID NO: 32 - protein, 448 aa, artificial sequence
  synthetic
QVQLQQSGPELVKPGASVTISCKASDYSFTNYYIHWVKQRPGQGLEWIGWIYPGNVITKYHEKFKGKAILTADTSSTTAYMQLNSLTSEDSAVYFCARSRATGYFDYWGQGTTLTVSSASTKGPSVFPLAPSSKSTSGGTAALGCLVKDYFPEPVTVSWNSGALTSGVHTFPAVLQSSGLYSLSSVVTVPSSSLGTQTYICNVNHKPSNTKVDKKAEPKSCDKTHTCPPCPAPELLGGPSVFLFPPKPKDTLMISRTPEVTCVVVDVSHEDPEVKFNWYVDGVEVHNAKTKPREEQYNSTYRVVSVLTVLHQDWLNGKEYKCKVSNKALPAPIEKTISKAKGQPREPQVYTLPPSRDELTKNQVSLTCLVKGFYPSDIAVEWESNGQPENNYKTTPPVLDSDGSFFLYSKLTVDKSRWQQGNVFSCSVMHEALHNHYTQKSLSLSPGK

SEQ ID NO: 33 - protein, 448 aa, artificial sequence
  synthetic
QVQLVQSGAEVKKPGASVKVSCKASDYSFTNYYIHWVRQAPGQGLEWMGWIYPGNVITKYHEKFKGRVTMTADTSTSTAYMELSSLRSEDTAVYYCARSRATGYFDYWGQGTLVTVSSASTKGPSVFPLAPSSKSTSGGTAALGCLVKDYFPEPVTVSWNSGALTSGVHTFPAVLQSSGLYSLSSVVTVPSSSLGTQTYICNVNHKPSNTKVDKKAEPKSCDKTHTCPPCPAPELLGGPSVFLFPPKPKDTLMISRTPEVTCVVVDVSHEDPEVKFNWYVDGVEVHNAKTKPREEQYNSTYRVVSVLTVLHQDWLNGKEYKCKVSNKALPAPIEKTISKAKGQPREPQVYTLPPSRDELTKNQVSLTCLVKGFYPSDIAVEWESNGQPENNYKTTPPVLDSDGSFFLYSKLTVDKSRWQQGNVFSCSVMHEALHNHYTQKSLSLSPGK

SEQ ID NO: 34 - protein, 449 aa, artificial sequence
  synthetic
EVQLQQSGAELARPGASVMLSCKASGYTFTSYWMQWLKQRPGQGLEWIGAIYPGDGDTRYTQKFKGKATLTADKSSSTAYMQLSSLASEDSAVYYCVRDDGLYYAMDYWGQGTSVTVSSASTKGPSVFPLAPSSKSTSGGTAALGCLVKDYFPEPVTVSWNSGALTSGVHTFPAVLQSSGLYSLSSVVTVPSSSLGTQTYICNVNHKPSNTKVDKKAEPKSCDKTHTCPPCPAPELLGGPSVFLFPPKPKDTLMISRTPEVTCVVVDVSHEDPEVKFNWYVDGVEVHNAKTKPREEQYNSTYRVVSVLTVLHQDWLNGKEYKCKVSNKALPAPIEKTISKAKGQPREPQVYTLPPSRDELTKNQVSLTCLVKGFYPSDIAVEWESNGQPENNYKTTPPVLDSDGSFFLYSKLTVDKSRWQQGNVFSCSVMHEALHNHYTQKSLSLSPGK

SEQ ID NO: 35 - protein, 452 aa, artificial sequence
  synthetic
QIQLVQSGPELKKPGETVKISCKASGYTFTDYSMNWVKQAPGKGLKWMGWLNTETGEPIYADDFKGRFVFSLETSASTAYLEINNLNDEDTATYFCAREAIYYGTSYVLDYWGQGTSVTVSSASTKGPSVFPLAPSSKSTSGGTAALGCLVKDYFPEPVTVSWNSGALTSGVHTFPAVLQSSGLYSLSSVVTVPSSSLGTQTYICNVNHKPSNTKVDKKAEPKSCDKTHTCPPCPAPELLGGPSVFLFPPKPKDTLMISRTPEVTCVVVDVSHEDPEVKFNWYVDGVEVHNAKTKPREEQYNSTYRVVSVLTVLHQDWLNGKEYKCKVSNKALPAPIEKTISKAKGQPREPQVYTLPPSRDELTKNQVSLTCLVKGFYPSDIAVEWESNGQPENNYKTTPPVLDSDGSFFLYSKLTVDKSRWQQGNVFSCSVMHEALHNHYTQKSLSLSPGK

SEQ ID NO: 36 - protein, 452 aa, artificial sequence
  synthetic
QIQLVQSGSELKKPGASVKVSCKASGYTFTDYSMNWVRQAPGQGLEWMGWLNTETGEPIYADDFKGRFVFSLDTSVSTAYLQISSLKAEDTAVYFCAREAIYYGTSYVLDYWGQGTLVTVSSASTKGPSVFPLAPSSKSTSGGTAALGCLVKDYFPEPVTVSWNSGALTSGVHTFPAVLQSSGLYSLSSVVTVPSSSLGTQTYICNVNHKPSNTKVDKKAEPKSCDKTHTCPPCPAPELLGGPSVFLFPPKPKDTLMISRTPEVTCVVVDVSHEDPEVKFNWYVDGVEVHNAKTKPREEQYNSTYRVVSVLTVLHQDWLNGKEYKCKVSNKALPAPIEKTISKAKGQPREPQVYTLPPSRDELTKNQVSLTCLVKGFYPSDIAVEWESNGQPENNYKTTPPVLDSDGSFFLYSKLTVDKSRWQQGNVFSCSVMHEALHNHYTQKSLSLSPGK

SEQ ID NO: 37 - protein, 452 aa, artificial sequence
  synthetic
QVQLVQSGAEVKKPGASVKVSCKASGYTFTDYSMNWVRQAPGQRLEWMGWLNTETGEPIYADDFKGRVTITRDTSASTAYMELSSLRSEDTAVYYCAREAIYYGTSYVLDYWGQGTLVTVSSASTKGPSVFPLAPSSKSTSGGTAALGCLVKDYFPEPVTVSWNSGALTSGVHTFPAVLQSSGLYSLSSVVTVPSSSLGTQTYICNVNHKPSNTKVDKKAEPKSCDKTHTCPPCPAPELLGGPSVFLFPPKPKDTLMISRTPEVTCVVVDVSHEDPEVKFNWYVDGVEVHNAKTKPREEQYNSTYRVVSVLTVLHQDWLNGKEYKCKVSNKALPAPIEKTISKAKGQPREPQVYTLPPSRDELTKNQVSLTCLVKGFYPSDIAVEWESNGQPENNYKTTPPVLDSDGSFFLYSKLTVDKSRWQQGNVFSCSVMHEALHNHYTQKSLSLSPGK

SEQ ID NO: 38 - protein, 214 aa, artificial sequence
  synthetic
DIQMTQTTSSLSASLGDRVTISCRASQDIRNYLNWFQQKPDGTIKLLIYYTSRLHSGVPSRFSGSGSGTDYSLTISNLEQEDMATYFCQQFNTLPWTFGGGTKLEIKRTVAAPSVFIFPPSDEQLKSGTASVVCLLNNFYPREAKVQWKVDNALQSGNSQESVTEQDSKDSTYSLSSTLTLSKADYEKHKVYACEVTHQGLSSPVTKSFNRGEC

SEQ ID NO: 39 - protein, 214 aa, artificial sequence
  synthetic
DIQMTQSPSSLSASVGDRVTITCRASQDIRNYLNWYQQKPGKAPKLLIYYTSRLHSGVPSRFSGSGSGTDYTLTISSLQPEDFATYYCQQFNTLPWTFGGGTKVEIKRTVAAPSVFIFPPSDEQLKSGTASVVCLLNNFYPREAKVQWKVDNALQSGNSQESVTEQDSKDSTYSLSSTLTLSKADYEKHKVYACEVTHQGLSSPVTKSFNRGEC

SEQ ID NO: 40 - protein, 215 aa, artificial sequence
  synthetic
QIVLTQSPTIMSASLGERVTMTCTASSSVSSSYLHWYQQKPGSSPKLWIYSTSNLASGVPARFSGSGSGTSYSLTISSMEAEDAATYYCHQYHRSPPTFGGGTKLEIKRTVAAPSVFIFPPSDEQLKSGTASVVCLLNNFYPREAKVQWKVDNALQSGNSQESVTEQDSKDSTYSLSSTLTLSKADYEKHKVYACEVTHQGLSSPVTKSFNRGEC

SEQ ID NO: 41 - protein, 218 aa, artificial sequence
  synthetic
DIVLTQSPASLAVSLGQRATISCRASESVEYYGTNFMQWYQQKPGQPPKLLIYSASNVESGVPARFSGSGSGTDFSLNIHPVEEDDIAVYFCQQSRKDPSTFGEGTNLEIKRTVAAPSVFIFPPSDEQLKSGTASVVCLLNNFYPREAKVQWKVDNALQSGNSQESVTEQDSKDSTYSLSSTLTLSKADYEKHKVYACEVTHQGLSSPVTKSFNRGEC

SEQ ID NO: 42 - protein, 218 aa, artificial sequence
  synthetic
DIVLTQSPASLAVSPGQRATITCRASESVEYYGTNFMQWYQQKPGQPPKLLIYSASNVESGVPARFSGSGSGTDFTLTINPVEANDTANYYCQQSRKDPSTFGQGTKLEIKRTVAAPSVFIFPPSDEQLKSGTASVVCLLNNFYPREAKVQWKVDNALQSGNSQESVTEQDSKDSTYSLSSTLTLSKADYEKHKVYACEVTHQGLSSPVTKSFNRGEC

SEQ ID NO: 43 - protein, 218 aa, artificial sequence
  synthetic
DIVLTQSPASLAVSPGQRATITCRASESVEYYGTNFMQWYQQKPGQPPKLLIYSASNVESGVPARFSGSGSGTDFTLTINPVEANDTANYFCQQSRKDPSTFGQGTKLEIKRTVAAPSVFIFPPSDEQLKSGTASVVCLLNNFYPREAKVQWKVDNALQSGNSQESVTEQDSKDSTYSLSSTLTLSKADYEKHKVYACEVTHQGLSSPVTKSFNRGEC

SEQ ID NO: 44 - protein, 218 aa, artificial sequence
  synthetic
DIVLTQSPASLAVSPGQRATITCRASESVEYYGTNFMQWYQQKPGQPPKLLIYSASNVESGVPARFSGSGSGTDFTLTINPVEAQDTANYFCQQSRKDPSTFGQGTKLEIKRTVAAPSVFIFPPSDEQLKSGTASVVCLLNNFYPREAKVQWKVDNALQSGNSQESVTEQDSKDSTYSLSSTLTLSKADYEKHKVYACEVTHQGLSSPVTKSFNRGEC

SEQ ID NO: 45 - DNA, 354 bp, artificial sequence
  synthetic
caggtccagctgcagcagtctggacctgagctggtgaagcctggggcgtcagtgacgatatcctgcaaggcttctgattattccttcacaaactactatatccactgggtgaagcagaggcctggacagggacttgaatggattggatggatatatcctggaaatgttattactaagtaccatgagaagtttaagggcaaggccatactgactgcagacacatcctccaccacagcctacatgcagctcaacagcctgacctctgaagactctgcggtctatttctgtgcaagatctagggctacgggctactttgactactggggccaaggcaccactctcacagtctcctca

SEQ ID NO: 46 - DNA, 321 bp, artificial sequence
  synthetic
gatatccagatgacacagactacatcctccctgtctgcctctctgggagacagagtcaccatcagttgcagggcaagtcaggacattcgcaattatttaaactggtttcagcagaaaccagatggaactattaaactcctgatctactacacatcaagattacactcaggggtcccatcaaggttcagtggcagtgggtctggaacagattattctctcaccattagcaacctggagcaagaagatatggccacttatttttgccaacaatttaatacgcttccgtggacgttcggtggaggcaccaagctggaaatcaaa

SEQ ID NO: 47 - DNA, 354 bp, artificial sequence
  synthetic
caggtgcagctggtgcagtcaggagcagaagtgaagaagccaggcgcaagcgtgaaggtgtcttgcaaggccagcgactacagcttcaccaactactacatccattgggtccggcaggctccaggacagggactcgagtggatgggttggatctaccccggcaacgtgatcaccaagtaccacgagaagttcaagggccgcgtgaccatgaccgcagacaccagcaccagcaccgcatacatggagctgagcagcctgaggagcgaggataccgccgtgtactattgcgccaggagcagagccaccggatacttcgactattggggccagggaacactggtgacagtgtctagc

SEQ ID NO: 48 - DNA, 321 bp, artificial sequence
  synthetic
gacatccagatgacccagagccctagcagcctgagcgctagcgtgggagatagagtgaccatcacctgtagagccagccaggacatccggaactacctgaattggtaccagcagaagcccggcaaggcccctaagctgctgatctactacaccagcagactgcacagcggagtgccttctagattcagcggcagcggaagcggcacagattacaccctgaccatcagcagcctgcagccagaggacttcgccacctactactgccagcagttcaacaccctgccttggaccttcggcggaggcaccaaggtggagatcaag

SEQ ID NO: 49 - DNA, 358 bp, artificial sequence
  synthetic
gaggttcagctgcagcagtctggggctgagctggcaagacctggggcttcagtgatgttgtcctgcaaggcttctggctacacctttactagctactggatgcagtggctaaaacagaggcctggacagggtctggaatggattggggctatttatcctggagatggtgatactaggtacactcagaagttcaagggcaaggccacattgactgcagataaatcctccagcacagcctacatgcaactcagcagcttggcatctgaggactctgcggtctattactgtgtaagagacgacggcctttactatgctatggactactggggtcaaggaacctcagtcaccgtctcctcag

SEQ ID NO: 50 - DNA, 324 bp, artificial sequence
  synthetic
caaattgttctcacccagtctccaacaatcatgtctgcatctctaggggaacgggtcaccatgacctgcactgccagctcaagtgtaagttccagttacttgcactggtaccagcagaagccaggatcctcccccaaactctggatttatagcacatccaacctggcttctggagtcccagctcgcttcagtggcagtgggtctgggacctcttactctctcacaatcagcagcatggaggctgaagatgctgccacttattactgccaccagtatcatcgttccccacccacgttcggaggggggaccaagctggaaataaaa

SEQ ID NO: 51 - DNA, 366 bp, artificial sequence
  synthetic
cagatccagttggtgcagtctggacctgagctgaaaaagcctggagagacagtcaagatctcctgcaaggcttctggttataccttcacagactattcaatgaactgggtgaagcaggctccaggaaagggtttaaagtggatgggctggctaaacactgagactggtgagccaatatatgcagatgacttcaagggacggtttgtcttctctttggaaacctctgccagcactgcctatttggagatcaacaacctcaatgatgaggacacggctacttatttctgtgctagagaagcaatctactatggcaccagctatgttctggactactggggtcaaggaacctcagtcaccgtctcctca

SEQ ID NO: 52 - DNA, 333 bp, artificial sequence
  synthetic
gacattgtgctgacccaatctccagcttctttggctgtgtctctaggacagagagccaccatctcctgcagagccagtgaaagtgttgaatattatggcacaaattttatgcagtggtaccaacagaaaccaggacagccacccaaactcctcatctattctgcatccaacgtagaatctggggtccctgccaggtttagtggcagtgggtctgggacagacttcagtctcaacatccatcctgtggaggaagatgatattgcagtgtatttctgtcaacaaagtaggaaggatccttcgacgttcggtgaaggcaccaacctggaaatcaaa

SEQ ID NO: 53 - DNA, 366 bp, artificial sequence
  synthetic
cagatccagctggtccagagcggcagcgagctgaagaaacccggcgccagcgtgaaggtgagctgcaaggccagcggctacaccttcaccgactacagcatgaactgggtgagacaagctcccggtcaaggtttagagtggatgggctggctgaacaccgagaccggcgagcccatctacgccgacgacttcaagggtcgtttcgtgttctctttagacaccagcgtgagcaccgcctatttacagatcagctctttaaaggccgaggacaccgccgtgtacttctgcgctcgtgaggccatctactacggcaccagctacgtgctggactactggggccaaggtacactggtgaccgtgagctcc

SEQ ID NO: 54 - DNA, 333 bp, artificial sequence
  synthetic
gacatcgtgctgacccagagccccgcttctttagctgtgagccccggtcagagagccaccatcacttgtcgtgccagcgagagcgtggagtactacggcaccaacttcatgcagtggtaccagcagaagcccggtcagccccccaagctgctgatctacagcgccagcaacgtcgagagcggagtgcccgctagatttagcggcagcggtagcggcacagacttcactttaaccatcaaccccgtggaggccaacgacaccgccaactactactgccagcagtctcgtaaggaccccagcaccttcggccaaggtaccaagctggagatcaag

SEQ ID NO: 55 - DNA, 366 bp, artificial sequence
  synthetic
caagttcagctggtgcagtccggcgccgaagtgaagaaacccggcgccagcgtgaaggtgagctgcaaggccagcggctacaccttcaccgactacagcatgaactgggtgagacaagctcccggtcagagactggagtggatgggctggctgaacaccgagaccggcgagcccatctacgccgacgacttcaagggtcgtgtgaccatcactcgtgacaccagcgccagcaccgcctacatggagctgagctctttaaggagcgaggacaccgccgtctactattgcgctcgtgaggccatctactacggcacctcctacgtgctggactactggggccaaggtactttagtgaccgtgagcagc

SEQ ID NO: 56 - DNA, 332 bp, artificial sequence
  synthetic
acatcgtgctgacccagagccccgcttctttagctgtgagccccggtcagagagccaccatcacttgtcgtgccagcgagagcgtggagtactacggcaccaacttcatgcagtggtaccagcagaagcccggtcagccccccaagctgctgatctacagcgccagcaacgtcgagagcggagtgcccgctagatttagcggcagcggtagcggcacagacttcactttaaccatcaaccccgtggaggccaacgacaccgccaactacttctgccagcagtctcgtaaggaccccagcaccttcggccaaggtaccaagctggagatcaag

SEQ ID NO: 57 - DNA, 332 bp, artificial sequence; identical to SEQ ID NO: 56
  synthetic

SEQ ID NO: 58 - protein, 119 aa, artificial sequence
  synthetic
QVTLKESGPALVKPTQTLTLTCTFSGFSLSTSGMGVGWIRQPPGKALEWLAHIWWDDDKFYNPSLKSRLTISKDTSKNQVVLTMTNMDPVDTATYYCARLTGTRYFDYWGQGTTVTVSS

SEQ ID NO: 59 - protein, 106 aa, artificial sequence
  synthetic
DVQMTQSPSSLSASVGDRVTITCKASQDINKFIAWYQQKPGKAPKLLIHYTSTLQPGIPSRFSGSGSGRDYTFTISSLQPEDIATYYCLQYGNLWTFGGGTKVEIK

SEQ ID NO: 60 - protein, 461 aa, artificial sequence
  synthetic
MAPVAVWAALAVGLELWAAAHALPAQVAFTPYAPEPGSTCRLREYYDQTAQMCCSKCSPGQHAKVFCTKTSDTVCDSCEDSTYTQLWNWVPECLSCGSRCSSDQVETQACTREQNRICTCRPGWYCALSKQEGCRLCAPLRKCRPGFGVARPGTETSDVVCKPCAPGTFSNTTSSTDICRPHQICNVVAIPGNASMDAVCTSTSPTRSMAPGAVHLPQPVSTRSQHTQPTPEPSTAPSTSFLLPMGPSPPAEGSTGDFALPVGLIVGVTALGLLIIGVVNCVIMTQVKKKPLCLQREAKVPHLPADKARGTQGPEQQHLLITAPSSSSSSLESSASALDRRAPTRNQPQAPGVEASGAGEARASTGSSDSSPGGHGTQVNVTCIVNVCSSSDHSSQCSSQASSTMGDTDSSPSESPKDEQVPFSKEECAFRSQLETPETLLGSTEEKPLPLGVPDAGMKPS

SEQ ID NO: 61 - protein, 463 aa, artificial sequence
  synthetic
MAPAAVWAALAVGLELWAAGHALPAQVAFTPYAPEPGGTCRLREYYDQTAQMCCSKCPPGQHAKVFCTKTSDTVCDSCEDSTYTQLWNWVPECLSCGSRCSSDQVETQACTREQNRICTCRPGWYCALSKQEGCRLCAQLRKCRPGFGVARPGTETSDVVCKPCAPGTFSNTTSSTDICRPHQICHVVAIPGNASMDAVCTSTSPTRSMAPGAVHLPQPVSTRSQHTQPTPAPSTAPGTSFLLPVGPSPPAEGSTGDIVLPVGLIVGVTALGLLIIGVVNCVIMTQVKKKPLCLQRETKVPHLPADKARGAQGPEQQHLLTTVPSSSSSSLESSASALDRRAPTRNQPQAPGAEKASGAGEARASTGSSADSSPGGHGTQVNVTCIVNVCSSSDHSSQCSSQASSTMGDTDASPSGSPKDEQVPFSKEESAFRSQLETPETLLGSTEEKPLPLGVPDAGMKPS

SEQ ID NO: 62 - protein, 330 aa, artificial sequence
  synthetic
ASTKGPSVFPLAPSSKSTSGGTAALGCLVKDYFPEPVTVSWNSGALTSGVHTFPAVLQSSGLYSLSSVVTVPSSSLGTQTYICNVNHKPSNTKVDKKAEPKSCDKTHTCPPCPAPELLGGPSVFLFPPKPKDTLMISRTPEVTCVVVDVSHEDPEVKFNWYVDGVEVHNAKTKPREEQYNSTYRVVSVLTVLHQDWLNGKEYKCKVSNKALPAPIEKTISKAKGQPREPQVYTLPPSRDELTKNQVSLTCLVKGFYPSDIAVEWESNGQPENNYKTTPPVLDSDGSFFLYSKLTVDKSRWQQGNVFSCSVMHEALHNHYTQKSLSLSPGK

SEQ ID NO: 63 - protein, 107 aa, artificial sequence [sequence omitted]

SEQ ID NO: 64 - protein, 122 aa, artificial sequence; identical to SEQ ID NO: 27
  synthetic

SEQ ID NO: 65 - protein, 111 aa, artificial sequence; identical to SEQ ID NO: 31
  synthetic

SEQ ID NO: 66 - protein, 452 aa, artificial sequence; identical to SEQ ID NO: 36
  synthetic

SEQ ID NO: 67 - protein, 218 aa, artificial sequence; identical to SEQ ID NO: 44
  synthetic

SEQ ID NO: 68 - protein, 366 aa, artificial sequence
  synthetic
CAGATCCAGCTGGTCCAGAGCGGCAGCGAGCTGAAGAAACCCGGCGCCAGCGTGAAGGTGAGCTGCAAGGCCAGCGGCTACACCTTCACCGACTACAGCATGAACTGGGTGAGACAAGCTCCCGGTCAAGGTTTAGAGTGGATGGGCTGGCTGAACACCGAGACCGGCGAGCCCATCTACGCCGACGACTTCAAGGGTCGTTTCGTGTTCTCTTTAGACACCAGCGTGAGCACCGCCTATTTACAGATCAGCTCTTTAAAGGCCGAGGACACCGCCGTGTACTTCTGCGCTCGTGAGGCCATCTACTACGGCACCAGCTACGTGCTGGACTACTGGGGCCAAGGTACACTGGTGACCGTGAGCTCC

SEQ ID NO: 69 - protein, 333 aa, artificial sequence
  synthetic
GACATCGTGCTGACCCAGAGCCCCGCTTCTTTAGCTGTGAGCCCCGGTCAGAGAGCCACCATCACTTGTCGTGCCAGCGAGAGCGTGGAGTACTACGGCACCAACTTCATGCAGTGGTACCAGCAGAAGCCCGGTCAGCCCCCCAAGCTGCTGATCTACAGCGCCAGCAACGTCGAGAGCGGAGTGCCCGCTAGATTTAGCGGCAGCGGTAGCGGCACAGACTTCACTTTAACCATCAACCCCGTGGAGGCCAACGACACCGCCAACTACTTCTGCCAGCAGTCTCGTAAGGACCCCAGCACCTTCGGCCAAGGTACCAAGCTGGAGATCAAG